European Patent Application EP 4 674 428 A1, published January 7, 2026. Title: Composition for use in treatment and/or prevention of complications of chronic kidney disease, agent for inhibiting progression of renal damage, agent for inhibiting progression of sarcopenia, and agent for inhibiting progression of anemia. Applicant: TOHOKU UNIVERSITY. The sequence listing filed with the application follows.

SEQUENCE LISTING (8 sequences)

SEQ ID NO: 1 - DNA, 20 bp, synthetic construct
  source 1..20: mol_type = other DNA
tgactggaagagcggagagt

SEQ ID NO: 2 - DNA, 20 bp, synthetic construct
  source 1..20: mol_type = other DNA
gaatccatcggtcatgctct

SEQ ID NO: 3 - DNA, 24 bp, synthetic construct
  source 1..24: mol_type = other DNA
gtgaaactggtgaacgtggctcta

SEQ ID NO: 4 - DNA, 20 bp, synthetic construct
  source 1..20: mol_type = other DNA
aggacctggatgcccacttg

SEQ ID NO: 5 - DNA, 20 bp, synthetic construct
  source 1..20: mol_type = other DNA
ggctattccttcgtgatgca

SEQ ID NO: 6 - DNA, 21 bp, synthetic construct
  source 1..21: mol_type = other DNA
ctaaactcttccagacaggac

SEQ ID NO: 7 - DNA, 24 bp, synthetic construct
  source 1..24: mol_type = other DNA
ttcagtggccaatggaagactcct

SEQ ID NO: 8 - DNA, 24 bp, synthetic construct
  source 1..24: mol_type = other DNA
agggcagttccacaacgtcatact